European Patent Application EP 4 349 366 A1, published April 10, 2024. Title: Pharmaceutical composition. Applicant: MIE UNIVERSITY. The sequence listing filed with the application follows.

SEQUENCE LISTING (14 sequences)

SEQ ID NO: 1 - protein, 9 aa, Artificial Sequence
  mutated ERK2 peptide
QYIHSANVL

SEQ ID NO: 2 - protein, 37 aa, Artificial Sequence
  long chain peptide
NDHIAYFLYQILRGLQYIHSANVLHRDLKPSNLLLNT

SEQ ID NO: 3 - protein, 17 aa, Artificial Sequence
  epitope sequence
RGLQYIHSANVLHRDLK

SEQ ID NO: 4 - protein, 9 aa, Artificial Sequence
  p25-33
EGSRNQDWL

SEQ ID NO: 5 - protein, 38 aa, Artificial Sequence
  gp100 TRP2 TRP1_6Y
SVYDFFVWLYYYYYYTWHRYHLLYYYYYYEGSRNQDWL

SEQ ID NO: 6 - protein, 9 aa, Artificial Sequence
  TRP2
SVYDFFVWL

SEQ ID NO: 7 - protein, 8 aa, Artificial Sequence
  TRP1
TWHRYHLL

SEQ ID NO: 8 - protein, 29 aa, Artificial Sequence
  MAGE-A4
AMEGDSASEEEIWEELGVMGVYDGREHTV

SEQ ID NO: 9 - protein, 10 aa, Artificial Sequence
  MAGE4
GVYDGREHTV

SEQ ID NO: 10 - protein, 20 aa, Artificial Sequence
  MAGE-A4 CD8 epitope tandem
GVYDGREHTVGVYDGREHTV

SEQ ID NO: 11 - DNA, 1580 bp, Artificial Sequence
  mMAGEzG CAR
gcggccgcagatccatgagtgtgcccactcaggtcctggggttgctgctgctgtggcttacaggtgccagatgtcaggtccagctggtacagtctggggctgaggtgaagaagcctgggtcctcggtgaaggtctcctgcaaggcttctggaggcaccttcagcagctatgctatcagctgggtgcgacaggcccctggacaagggcttgagtggatgggagggatcatccctatctttggtacagcaaactacgcacagaagttccagggcagagtcacgattaccgcggacaaatccacgagcacagcctacatggagctgagcagcctgagatctgaggacacggccgtgtattactgtgcgagatccccccggcgggcatatcatgatgcttttgatatctggggccaagggacaatggtcaccgtctcttcaggtggaggcggttcaggcggaggtggcagcggcggtggcgggagttcctatgagctgactcagccaccctcgatgtcagtggccccaggaaagacggccagcattacctgtggcggagaccatattggaagtaaaagtgttcactggtaccagcagaagccaggccaggcccctgtactggtcgtctatgatgatagcgaccggccctcagggatccctgagcgattctctggctccaactctgggaacacagccactctgaccatcagcgggacccaggctatggatgaggctgactattactgtctggcgtgggacagcagcactgcgatcttcggcggagggaccaagctgaccgtcctagcggcgcgccagatcagcaactcggtgatgtacttcagttctgtcgtgccagtccttcagaaagtgaactctactactaccaagccagtgctgcgaactccctcacctgtgcaccctaccgggacatctcagccccagagaccagaagattgtcggccccgtggctcagtgaaggggaccggattggactctagattttgggcactggtcgtggttgctggagtcctgttttgttatggcttgctagtgacagtggctctttgtgttatctggacaaatctgagagcaaaattcagcaggagtgcagagactgctgccaacctgcaggaccccaaccagctctacaatgagctcaatctagggcgaagagaggaatatgacgtcttggagaagaagcgggctcgggatccagagatgggaggcaaacagcagaggaggaggaacccccaggaaggcgtatacaatgcactgcagaaagacaagatggcagaagcctacagtgagatcggcacaaaaggcgagaggcggagaggcaaggggcacgatggcctttaccagggtctcagcactgccaccaaggacacctatgatgccctgcatatgcagaccctggcccctcgcaggaggcaacacatgtgtcctcgagagacccagccattcgcggaggtgcagttgtcagctgaggatgcttgcagcttccagttccctgaggaggaacgcggggagcagacagaagaaaagtgtcatctggggggtcggtggccataatcgattctcgag

SEQ ID NO: 12 - DNA, 1556 bp, Artificial Sequence
  mMAGE 28z CAR
gcggccgcagatccatgagtgtgcccactcaggtcctggggttgctgctgctgtggcttacaggtgccagatgtcaggtccagctggtacagtctggggctgaggtgaagaagcctgggtcctcggtgaaggtctcctgcaaggcttctggaggcaccttcagcagctatgctatcagctgggtgcgacaggcccctggacaagggcttgagtggatgggagggatcatccctatctttggtacagcaaactacgcacagaagttccagggcagagtcacgattaccgcggacaaatccacgagcacagcctacatggagctgagcagcctgagatctgaggacacggccgtgtattactgtgcgagatccccccggcgggcatatcatgatgcttttgatatctggggccaagggacaatggtcaccgtctcttcaggtggaggcggttcaggcggaggtggcagcggcggtggcgggagttcctatgagctgactcagccaccctcgatgtcagtggccccaggaaagacggccagcattacctgtggcggagaccatattggaagtaaaagtgttcactggtaccagcagaagccaggccaggcccctgtactggtcgtctatgatgatagcgaccggccctcagggatccctgagcgattctctggctccaactctgggaacacagccactctgaccatcagcgggacccaggctatggatgaggctgactattactgtctggcgtgggacagcagcactgcgatcttcggcggagggaccaagctgaccgtcctagcggcgcgccagatcagcaactcggtgatgtacttcagttctgtcgtgccagtccttcagaaagtgaactctactactaccaagccagtgctgcgaactccctcacctgtgcaccctaccgggacatctcagccccagagaccagaagattgtcggccccgtggctcagtgaaggggaccggattggactctagattttgggcactggtcgtggttgctggagtcctgttttgttatggcttgctagtgacagtggctctttgtgttatctggacaaatagtagaaggaacagactccttcaaagtgactacatgaacatgactccccggaggcctgggctcactcgaaagccttaccagccctacgcccctgccagagactttgcagcgtaccgccccctgagagcaaaattcagcaggagtgcagagactgctgccaacctgcaggaccccaaccagctctacaatgagctcaatctagggcgaagagaggaatatgacgtcttggagaagaagcgggctcgggatccagagatgggaggcaaacagcagaggaggaggaacccccaggaaggcgtatacaatgcactgcagaaagacaagatggcagaagcctacagtgagatcggcacaaaaggcgagaggcggagaggcaaggggcacgatggcctttaccagggtctcagcactgccaccaaggacacctatgatgccctgcatatgcagaccctggcccctcgctaatcgattctcgag

SEQ ID NO: 13 - DNA, 1979 bp, Artificial Sequence
  MAGE-A4 expression vector
gcggccgcaccaccatgagctccgagcagaagagccagcactgcaaacccgaggaaggcgttgaagcccaggaagaagcactgggtctggttggagcacaagctcccactaccgaagaacaggaggctgccgtttccagtagctctccccttgtgccaggaaccctggaagaggtccctgctgccgagtctgccggtcctcctcagagtcctcaaggcgcaagcgccttgcccacgaccatcagctttacgtgctggagacaacccaatgaaggatcaagctctcaggaggaagaaggcccatcaacatctccggatgcagaatcactctttcgcgaggcactcagcaacaaagtggacgaattggcccatttccttctgcggaagtacagggctaaagaactggtgacaaaggcggaaatgctggagagggtgatcaagaactacaagcggtgtttcccagtgatcttcggcaaagcatccgagagtctgaagatgatctttggcattgacgtgaaggaggtcgatccagcctccaacacctataccctggtgacttgtctcgggctctcctatgatgggcttttgggtaacaaccagatattccccaaaacagggctgctgatcattgtgctgggaaccatagccatggagggcgatagtgccagcgaagaagagatttgggaggagctgggagtgatgggtgtatatgacggacgagagcacactgtctatggcgagcctcggaaactcctgactcaggactgggtccaggagaattacctggagtatcgacaggtaccagggtcaaatccggctcgctacgagtttctttggggccctcgtgctttggcggagacatcctacgtcaaggtgctggagcatgtggtaagggtgaatgcgagagttcgcattgcctacccatctctgagagaggccgctctcctggaggaagaggaaggggttatcgatggaagcggagccacgaacttctctctgttaaagcaagcaggagatgttgaagaaaaccccgggcctatgaggagggctggagccgcctgttccgccatggatcgactgcgtttgctgcttctgctcctgctccttctgggtgtaagctttggaggagccaaagagacatgcagcactggcatgtatacccacagtggagaatgctgcaaggcatgcaacctcggcgaaggagttgctcagccttgtggcgcaaaccagactgtgtgtgaaccctgtctggacagtgtgacattcagcgatgtggtgtctgccaccgagccatgcaagccatgtaccgagtgtctgggtctgcaatccatgtctgcaccttgcgtggaagctgatgacgccgtttgtcgctgtagttacggttactatcaggacgaggaaacaggcagatgtgaggcttgcagcgtttgtggtgtagggtctggactggtgttctcctgccaggataagcagaatacagtgtgcgaagagtgtcccgaaggcacctatagcgatgaggccaatcacgtcgatccctgcctgccgtgtactgtctgcgaggatacagagcgccaattgcgcgaatgcacaccatgggccgatgcggagtgtgaggagatcccaggaaggtggattacgcggtctacccctcccgagggcagtgacgtaaccacaccctcaacccaggaacctgaggcaccaccggagcgggaccttatcgcgtcaaccgtcgctgacaccgtcacgacagtgatgggttctagccagccagtcgtgactagaggcactgcggacaacttgattccagtgtactgctctattctggctgccgtcgtcgttggcctcgtggcgtatatcgctttcaaacgatggaattcctgcaaacagaacaagcaaggggccaactcaagacccgtgaatcaaactcctcctcccgaaggggagaaactgcactctgatagcgggatatcctaactcgag

SEQ ID NO: 14 - DNA, 1451 bp, Artificial Sequence
  HHD A0201 Eexpression vector
gcggccgcaccaccatggccgtaatggctcctaggactctggtgctccttcttagtggagctttggctctgacccagacctgggccattcagcggactcccaagatacaggtgtacagcaggcatcccgctgagaatgggaaaagcaacttcctgaactgctatgtgagcggatttcacccatcagacatcgaagtggatctgttgaagaatggggagcggattgagaaggtcgagcattccgacctgtcattcagcaaagactggagcttttacctcctgtactataccgagtttacacccacagagaaggatgaatatgcatgccgagtgaatcacgttacgctgtctcagccaaagatcgtaaagtgggaccgggatatgggcggtggagggtcaggcggtggcggttcaggaggaggtgggagcggaagtcattccatgcgttacttcttcacatccgtgtcaagacctggcagaggggagccacgcttcatcgcagtcggctacgtcgatgatacccagttcgtccgctttgactctgacgcagccagtcagcgtatggaaccgcgtgcaccctggattgaacaggaaggccctgagtattgggatggggagactaggaaggtgaaagcccatagccagacacaccgagtcgaccttgggacgctgagaggatactacaaccagtccgaagctgggagtcacaccgttcagcgaatgtatggctgcgacgtaggctccgattggagattcctgaggggctatcaccagtacgcatacgatggtaaggactatatcgccctcaaagaggatctgcggtcctggacagccgctgacatggccgcgcaaacaacgaagcacaaatgggaggctgcgcatgtggccgagcaactgagggcctacctggagggaacttgtgtggagtggttgcgcagatacctggagaacggcaaggaaactctccaacgcaccgactctccgaaggcacatgtgactcaccacccaaggagtaagggtgaagtgaccttgcggtgttgggcactgggattctatcccgcagacatcacactgacctggcaactgaatggggaagaactgacccaggacatggagctcgtggagacaagaccagccggagatgggacatttcagaaatgggcgtctgttgttgtccctctcggcaaggagcagaactacacctgtcgcgtataccacgaagggttgcccgaacccctgaccctgcgatgggaacctccacctagcactgattcctatatggtgattgtggccgtccttggcgttctgggagctatggccatcataggtgctgtggttgcctttgtcatgaaaaggcgcagaaacactggtggcaaaggcggcgactatgctctcgcccctggaagccaatctagcgagatgtctcttcgggattgcaaagcttgactcgag